European Patent Application EP 4 279 586 A1, published November 22, 2023. Title: Engineered microorganisms expressing acetoacetyl-CoA reductase variants and method for improving the yield of PHA. Applicant: Shenzhen Bluepha Biosciences Co., Ltd. The sequence listing filed with the application follows.

SEQUENCE LISTING (52 sequences)

SEQ ID NO: 1 - DNA, 4235 bp, Artificial Sequence
  Laboratory synthesis
gtgacgcttgcatgagtgccggcgtgcgtcatgcacggcgccggcaggcctgcaggttccctcccgtttccattgaaaggactacacaatgactgacgttgtcatcgtatccgccgcccgcaccgcggtcggcaagtttggcggctcgctggccaagatcccggcaccggaactgggtgccgtggtcatcaaggccgcgctggagcgcgccggcgtcaagccggagcaggtgagcgaagtcatcatgggccaggtgctgaccgccggttcgggccagaaccccgcacgccaggccgcgatcaaggccggcctgccggcgatggtgccggccatgaccatcaacaaggtgtgcggctcgggcctgaaggccgtgatgctggccgccaacgcgatcatggcgggcgacgccgagatcgtggtggccggcggccaggaaaacatgagcgccgccccgcacgtgctgccgggctcgcgcgatggtttccgcatgggcgatgccaagctggtcgacaccatgcaccgctcgtcacatcctgttgcgttcactggaatcccagtatagactttgacctgcgagcaagctgtcaccggatgtgctttccggtctgatgagtccgtgaggacgaaacagcctctacaaataattttgtttaatgtggttatgtgcgttaaggaggtttaacgatgcgtaaaggcgaagagctgttcactggtgtcgtccctattctggtggaactggatggtgatgtcaacggtcataagttttccgtgcgtggcgagggtgaaggtgacgcaactaatggtaaactgacgctgaagttcatctgtactactggtaaactgccggtaccttggccgactctggtaacgacgctgacttatggtgttcagtgctttgctcgttatccgaaccatatgaagcagcatgacttcttcaagtccgccatgccggaaggctatgtgcaggaacgcacgatttcctttaaggatgacggcacgtacaaaacgcgtgcggaagtgaaatttgaaggcgataccctggtaaaccgcattgagctgaaaggcattgactttaaagaagacggcaatatcctgggccataagctggaatacaattttaacagccacaatgtttacatcaccgccgataaacaaaaaaatggcattaaagcgaattttaaaattcgccacaacgtggaggatggcagcgtgcagctggctgatcactaccagcaaaacactccaatcggtgatggtcctgttctgctgccagacaatcactatctgagcacgcaaagcgttctgtctaaagatccgaacgagaaacgcgatcatatggttctgctggagttcgtaaccgcagcgggcatcacgcatggtatggatgaactgtacaaataatcgtcactccaccggtgctacgaggccctttcgtcttcaagaattctcatgtttgacagcttatcatcgataagctttaatgcggtagtttatcacagttaaattgctaacgcagtcaggcaccgtgtatgaaatctaacaatgcgctcatcgtcatcctcggcaccgtcaccctggatgctgtaggcataggcttggttatgccggtactgccgggcctcttgcgggatatcgtccattccgacagcatcgccagtcactatggcgtgctgctagcgctatatgcgttgatgcaatttctatgcgcacccgttctcggagcactgtccgaccgctttggccgccgcccagtcctgctcgcttcgctacttggagccactatcgactacgcgatcatggcgaccacacccgtcctgtggatcctctacgccggacgcatcgtggccggcatcaccggcgccacaggtgcggttgctggcgcctatatcgccgacatcaccgatggggaagatcgggctcgccacttcgggctcatgagcgcttgtttcggcgtgggtatggtggcaggccccgtggccgggggactgttgggcgccatctccttgcatgcaccattccttgcggcggcggtgctcaacggcctcaacctactactgggctgcttcctaatgcaggagtcgcataagggagagcgtcgaccgatgcccttgagagccttcaacccagtcagctccttccggtgggcgcggggcatgactatcgtcgccgcacttatgactgtcttctttatcatgcaactcgtaggacaggtgccggcagcgctctgggtcattttcggcgaggaccgctttcgctggagcgcgacgatgatcggcctgtcgcttgcggtattcggaatcttgcacgccctcgctcaagccttcgtcactggtcccgccaccaaacgtttcggcgagaagcaggccattatcgccggcatggcggccgacgcgctgggctacgtcttgctggcgttcgcgacgcgaggctggatggccttccccattatgattcttctcgcttccggcggcatcgggatgcccgcgttgcaggccatgctgtccaggcaggtagatgacgaccatcagggacagcttcaaggatcgctcgcggctcttaccagcctaacttcgatcactggaccgctgatcgtcacggcgatttatgccgcctcggcgagcacatggaacgggttggcatggattgtaggcgccgccctataccttgtctgcctccccgcgttgcgtcgcggtgcatggagccgggccacctcgacctgaatggaagccggcggcacctcgctaacggattcaccactccaagaattggagccaatcaatttgacttttgtccttttccgctgcataaccctgcttcggggtcattatagcgattttttcggtatatccatcctttttcgcacgatatacaggattttgccaaagggttcgtgtagactttccttggtgtatccaacggcgtcagccgggcaggataggtgaagtaggcccacccgcgagcgggtgttccttcttcactgtcccttattcgcacctggcggtgctcaacgggaatcctgctctgcgaggctggccgtaggccggccgcgatgcaggtggctgctgaacccccagccggaactgaccccacaaggcccaagatccgcagttcaacctgttgatagtacgtactaagctctcatgtttcacgtactaagctctcatgtttaacgtactaagctctcatgtttaacgaactaaaccctcatggctaacgtactaagctctcatggctaacgtactaagctctcatgtttcacgtactaagctctcatgtttgaacaataaaattaatataaatcagcaacttaaatagcctctaaggttttaagttttataagaaaaaaaagaatatataaggcttttaaagcttttaaggtttaacggttgtggacaacaagccagggatgtaacgcactgagaagcccttagagcctctcaaagcaattttgagtgacacaggaacacttaacggctgacatggattaccctgttatccctaattaccctgttatccctaattaccctgttatccctaattaccctgttatccctaattaccctgttatccctaattaccctgttatccctaattaccctgttatccctaattaccctgttatccctatggtacccggccaagtctgcgggcgtgcccatgatgtagagcaccagcgccaccggcgccatgccatacatcaggaaggtggcaacgcctgccaccacgttgtgctcggtgatcgccatcatcagcgccacgtagagccagccaatggccacgatgtacatcaaaaattcatccttctcgcctatgctctggggcctcggcagatgcgagcgctgcataccgtccggtaggtcgggaagcgtgcagtgccgaggcggattcccgcattgacagcgcgtgcgttgcaaggcaacaatggactcaaatgtctcggaatcgctgacgattcccaggtttctccggcaagcatagcgcatggcgtctccatgcgagaatgtcgcgcttgccggataaaaggggagccgctatcggaatggacgcaagccacggccgcagcaggtgcggtcgagggcttccagccagttccagggcagatgtgccggcagaccctcccgctttgggggaggcgcaagccgggtccattcggatagcatctccccatgcaaagtgccggccagggcaatgcccggagccggttcgaatagtgacggcagagagacaatcaaatc

SEQ ID NO: 2 - DNA, 2887 bp, Artificial Sequence
  Laboratory synthesis
cgggcgtgcccatgatgtagagcaccagcgccaccggcgccatgccatacatcaggaaggtggcaacgcctgccaccacgttgtgctcggtgatcgccatcatcagcgccacgtagagccagccaatggccacgatgtacatcaaaaattcatccttctcgcctatgctctggggcctcggcagatgcgagcgctgcataccgtccggtaggtcgggaagcgtgcagtgccgaggcggattcccgcattgacagcgcgtgcgttgcaaggcaacaatggactcaaatgtctcggaatcgctgacgattcccaggtttctccggcaagcatagcgcatggcgtctccatgcgagaatgtcgcgcttgccggataaaaggggagccgctatcggaatggacgcaagccacggccgcagcaggtgcggtcgagggcttccagccagttccagggcagatgtgccggcagaccctcccgctttgggggaggcgcaagccgggtccattcggatagcatctccccatgcaaagtgccggccagggcaatgcccggagccggttcgaatagtgacggcagagagacaatcaaatcatgagccaaccatcttatggcccgctgttcgaggccctggcccactacaatgacaagctgctggccatggccaaggcccagacagagcgcaccgcccaggcgctgctgcagaccaatctggacgatctgggccaggtgctggagcagggcagccagcaaccctggcagctgatccaggcccagatgaactggtggcaggatcagctcaagctgatgcagcacaccctgctcaaaagcgcaggccagccgagcgagccggtgatcaccccggagcgcagcgatcgccgcttcaaggccgaggcctggagcgaacaacccatctatgactacctcaagcagtcctacctgctcaccgccaggcacctgctggcctcggtggatgccctggagggcgtcccccagaagagccgggagcggctgcgtttcttcacccgccagtacgtctctgccatggcccccagcaacttcctggccaccaaccccgagctgctcaagctgaccctggagtccggcggccagaacctggtgcgcggactggccctcttggccgaggatctggagcgcagcgccgatcagctcaacatccgcctgaccgacgaatccgccttcgagctcgggcgggatctggccctgaccccgggccgggtggtgcagcgcaccgagctctatgagctcattcagtacagcccgactaccgagacggtgggcaagacacctgtgctgatagtgccgcccttcatcaacaagtactacatcatggacatgcggccccagaactccctggtcgcctggctggtcgcccagggccagacggtattcatgatctcctggcgcaacccgggcgtggcccaggcccaaatcgatctcgacgactacgtggtggatggcgtcatcgccgccctggacggcgtggaggcggccaccggcgagcgggaggtgcacggcatcggctactgcatcggcggcaccgccctgtcgctcgccatgggctggctggcggcgcggcgccagaagcagcgggtgcgcaccgccaccctgttcactaccctgctggacttctcccagcccggggagcttggcatcttcatccacgagcccatcatagcggcgctcgaggcgcaaaatgaggccaagggcatcatggacgggcgccagctggcggtcagcttcagcctgctgcgggagaacagcctctactggaactactacatcgacagctacctcaagggtcagagcccggtggccttcgatctgctgcactggaacagcgacagcaccaatgtggcgggcaagacccacaacagcctgctgcgccgtctctacctggagaaccagctggtgaagggggagctcaagatccgcaacacccgcatcgatctcggcaaggtgaagacccctgtgctgctggtgtcggcggtggacgatcacatcgccctctggcagggcacctggcagggcatgaagctgtttggcggggagcagcgcttcctcctggcggagtccggccacatcgccggcatcatcaacccgccggccgccaacaagtacggcttctggcacaacggggccgaggccgagagcccggagagctggctggcaggggcgacgcaccagggcggctcctggtggcccgagatgatgggctttatccagaaccgtgacgaagggtcagagcccgtccccgcgcgggtcccggaggaagggctggcccccgcccccggccactatgtcaaggtgcggctcaaccccgtgtttgcctgcccaacagaggaggacgccgcatgacgcttgcatgagtgccggcgtgcgtcatgcacggcgccggcaggcctgcaggttccctcccgtttccattgaaaggactacacaatgactgacgttgtcatcgtatccgccgcccgcaccgcggtcggcaagtttggcggctcgctggccaagatcccggcaccggaactgggtgccgtggtcatcaaggccgcgctggagcgcgccggcgtcaagccggagcaggtgagcgaagtcatcatgggccaggtgctgaccgccggttcgggccagaaccccgcacgccaggccgcgatcaaggccggcctgccggcgatggtgccggccatgaccatcaacaaggtgtgcggctcgggcctgaaggccgtgatgctggccgccaacgcgatcatggcgggcgacgccgagatcgtggtggccggcggccaggaaaacatgagcgccgccccgcacgtgctgccgggctcgcgcgatggtttccgcatgggcgatgccaagctggtcgacaccatg

SEQ ID NO: 3 - DNA, 742 bp, Artificial Sequence
  Laboratory synthesis
atgaccagccgcgtggccctggtgaccggcggcaccggcggcatcggcaccgccatcgtgaagcgcctggcggccatgggccacaaggtggcgaccaactaccgcgacgaggccaaggccaaggcctgggccgacaagctgaagtcggagggcgtggacgtgctgctggtgaagggcgacgtgtcggacaccgccagcagcgaggccatgatcaaggagatcgagagcaagctgggcccgatcgacatcctgatcaacaacgcgggcatcacccgcgacaccaccttccacaagatgtcggccatgcagtggcaggaagtgatcaacaccaacctgaacagcgtgttcaacgtgacccgcccggtgatcgagggcatgcgcaaccgcaagtggggccgcatcatccagatctcgagcatcaacggccagaagggccagtacggccaggccaactacgcggccgccaaggcgggcatgcacggcttcaccatctcgctggcgcaggagaacgccaagttcggcatcaccgtgaacaccgtgagcccgggctacgtggccaccgagatggtgatggccgtgccggaggacgtgcgcaacaagatcgccgcccagatcccggtgggccgcctgggcgagccggaggagatcgcgtacgccatcgagttcttcgtgaaggacgaggccaagtggatcaccggcgccaacctggccatcaacggtggccagtacatgggctggtaag

SEQ ID NO: 4 - DNA, 729 bp, Artificial Sequence
  Laboratory synthesis
atggccaagcgcaacgccatcgtgaccggcggcacccgcggcatcggccacgccatcgcgatcgccctgaaggaagccggctgcaccgtggcggccacctaccacggcaacgacgaggccgcgaaggccttccacgaggaaaccggcgtggcggtgttcaagtgggacgtgggcgactacgacgcctgcaaggcgggcgtggccgagatcgagaaggcccacggcccgaccgacatcctggtgaacaacgccggcgtgacccgcgacggcttcttccacaagatgaccccggcccagtggcgcgaggtgatccgcgcggacctggactcggtgttcaacatgacccaccaggtgttcccgggcatgcgcgagcgcggcttcggccgcatcatcaacatctcgagcatcaacggccagaagggccagatgggccagaccaactacagcgccgcgaaggcgggcatgatcggcttcacccgcgccctggcccaggaaggcgcgttcaagggcgtgaccgtgaacgccgtggccccgggctacatcgccaccgacatggtggcgaagctggacgaaaccgtgctgcagaagatcgtggcccagatcccggtgggccgcctgggcgaggcggaggagatcgcgcgctgcgtggccttcctggccgacgacgcggccggcttcatcaccggcagcgtgctgaccgtgaacggtggccagtacatcgccgcgtaa

SEQ ID NO: 5 - DNA, 745 bp, Artificial Sequence
  Laboratory synthesis
atgacccagcacatcgccgtggtgaccggcgcctcgggcggcctgggcgaaaccatgtgcaaggcgatggtggaccagggccacaaggtggcgggcagctacctgccgggcaccgacgccgaggcgaagagctggcagcagtcgatgcaggcggccggctacgaggtggccatctacccgctggacgtgaccaactacgacaactgctgctcgttcatcgccaccgtggagaaggacctgggcccgatcagcatcctggtgaacaacgccggcatcacccgcgacgccccgctgaagcgcatgcagccgcagcagtggcaggacgtgctgcgcaccaacctggactcgatgtacaacatgtgccagccggtgttcgacgccatgtgcaaccgcggcttcggccgcatcgtgaacatctcgtcgctgaacggcgagcagggccagttcggccaggccaactacagcgcggccaaggccggcatctacggcttcaccaaggccatcgccaaggaaggcgcccgcaagggcgtgaccgtgaacgccgtgagcccgggcttcatcgacaccccgatggtgcgccaggtgccggagaacgtgctggagagcatcatctcgggcatcccggtgggccgcctgggccagccggaggagatcgcccgcgccgtggccttcctgaccgccgaggacgcgggctacatcaccggctcgaacatcagcgtgaacggcggcgagtacatgagctaag

SEQ ID NO: 6 - DNA, 724 bp, Artificial Sequence
  Laboratory synthesis
atgaagaacgtggccatcgtgaccggcggcacccgcggcatcggcctggagatcaccaaggccctgatcgcggagggctacaaggtggccgcgatctaccacggcaacgaggaagccgccaaggcctgcgaggccgaaaccggcgccaaggcgtacaagatcgacgtggccagctaccaggcctgccacgacggctgcgccaagatcgagcaggagatgggcccgatcagcctgctggtgaacaacgcgggcatcaccaaggacggcgtgctgcacaagatggccgaggaccagtggcacgcggtgatcgaaaccaacctgacctcgtgcttcaacatgtgccgcgcggtgatcaccggcatgcgcgagcgcgtgtacggccgcatcgtgaacatctcgagcatcaacggccagaagggccagttcggccagaccaactacagcgcggccaaggcgggcatgctgggcttcaccaaggccctggccctggagtcggcggccaagggcatcaccgtgaacgcgatctgcccgggctacatcgaaaccgagatgaccgccgcgatgaagcaggacgtgctggactcgatcgtgcgccagatcccggcggcccgcatgggcaagccgcaggagatcgccgacctggtggtgttcctggccagcgagaaggcgggcttcatcaacggcgccaccatgaccgccaacggtggccagtacatgatctaag

SEQ ID NO: 7 - DNA, 748 bp, Artificial Sequence
  Laboratory synthesis
atgaagaacagcaccggccgcgtggccctgatcaccggcagcaccggcggcatcggcaccgccctgtgcaagaagctgtgcgaggaaggcttccgcgtggtgggcaacttccgctgctgggagaaggcccaggcgatgcagaacaccctgcaggacgtgggctgcgaggtggacatgcgccagggcgacgtggcggacttcgacagcgtgggccgcatggtgcgcgccgtggagtcggagatcggcccgatcgacgtgctgatcaacaacgcgggcatcgcccgcgacgtgcgcttcaccaagatggagaaggccgactgggacgacgtgatgaacaccaacctgaacggcgtgttcaactgcacccgccacgtgatcgacggcatgatggcccgtcgctacggccgcatcatcaacatctcgagcatcaacggccagaagggccagttcggccagaccaactacagcgcggccaaggcgggcatccacggcttcaccaagagcctggccctggaggtggcgaagtacggcatcaccgtgaacaccatctcgccgggctacatcgaaaccgagatggtgatggccgtgccgcagaacatccgcgagcagatcgtggcccagatcccggtgggccgcatgggctacatcgaggaagtggccgaggcggtgagctacctggtgtcggacaagagcggcttcatcaccggctcgaacctgagcatcaacggtggccagcacatgtactaag

SEQ ID NO: 8 - DNA, 751 bp, Artificial Sequence
  Laboratory synthesis
atgtgcggcgacctgaagaacaaggtggccctggtgaccggcggcaccggcggcatcggcaccgcgatctgcgcccgcctgtcggacctgggctgccgcgtggccaccacctaccgcaaccgcgagaaggccgaggcctggcaggcccagatgaagcagagcggccaccaggtgaccatctacgcctgcgacgtgggcgactacgaggcctgcgtgcagctggccgaaaccatcgagaaggacctgggcccggtggacatcctggtgaacaacgcgggcatcacccgcgacaccaccctgaagaagatgaccccgggccactggcgcgaggtgatctgcgcggacctggactcggtgttcaacatgacccagccgctgctgccgcgcatggcggagcgcggctggggccgcgtgatcaacatctcgagcatcaacggccagaagggccagttcggccaggccaactacagcgcggccaaggcgggcatgcacggcttcaccatggcggccgcccaggaagtggcccgcaagggcgtgaccgtgaacaccatcagcccgggctacatcgcgaccgagatggtgatggccgtgccggaggaagtgcgcgacaagatcatcgcccagatcccggtgggccgcctgggccgtccggaggaagtggcccacgtggtggcgttcctggcctcggagcacgccggcttcatcaccggcgccaacttcgccgccaacggtggccagcacatgcactaag

SEQ ID NO: 9 - DNA, 742 bp, Artificial Sequence
  Laboratory synthesis
atgtcgcagcgcaccgccctggtgaccggcggcaccggcggcatcggcaccgccatcgtgcgctacctgagccgccagggccaccgcgtggcgaccaactaccgcgacgcggcccgcgcggaggagtggcgcaagcgcatggcggccgagggcatcgaggtgtgcctggtgccgggcgacgtggcggacccggccagcgccgaggcgatggtgcgcgccgtggaggccaagtgcggcccggtggagatcctggtgaacaacgccggcatcacccgcgacaccaccttccacaagatgacctaccagcagtggaccgacgtggtgaacaccaacctgaacgcgtgcttcaacgtgacccgcccggtgatcgagggcatgcgcgcccgcaagtggggccgcatcgtgcagatctcgagcatcaacggccagaagggccagtacggccaggccaactacgcggccgccaaggcgggcatgcacggcttcaccatcagcctggcccaggagaacgcccgcttcggcatcaccgtgaacaccgtgagcccgggctacgtggccaccgacatggtgatggccgtgccggaggaagtgcgcgagaagatcgtggcccagatcccggtgggccgcctgggcaagccggaggagatcgcccacgcggtggccttcttcaccaccgacgaggccagctggatcaccggcgccaacctggccatcaacggtggccactacatgggctggtaag

SEQ ID NO: 10 - DNA, 724 bp, Artificial Sequence
  Laboratory synthesis
atgagccgcgtggtggtggtgaccggcggcacccgcggcatcggcgaggagatctgcgtggagcacaaggcggccggctacaccgtggccgcgatctacggtggcaacgacgaggcggccaaggccttcaccgagcgcaccggcatcaacgcctacaagtgcgacgtgagcgactacgacgcgtgccaggaagccgtgcaggtgatcgagaaggagctgggcccggtggacatcctggtgaacaacgccggcatcacccgcgacggcgccatgcacaagatggacttcgagcgctggaacgcggtgatccagaccaacctgtcgagctgcttcaacatgtcgaaggcggtgatcgacggcatgcgcgagcgcgagttcggccgcatcgtgaacatcggctcggtgaacggccgcgccggccagtacggccaggtgaactacgcggccgccaagagcggcatccacggcttcaccaaggccctggccctggagggcgccagcaagggcatcaccgtgaacgccatcgccccgggctacgtgctgaccgacatggtgcgcgccgtgccgcagaaggtgctggacaagatcatcgccaccatcccggtgggccgcctgggcgacccgggcgacatcgcgcgcgccgtgatgttcctgaccagcgacggctcgggcttcgtgaccggcagcaccctggacgtgaacggtggccagcacatgtactaag

SEQ ID NO: 11 - DNA, 745 bp, Artificial Sequence
  Laboratory synthesis
atgcaggaccgcatcgccttcgtgaccggcggcaccggcggcatcggcagcgcgatctgcaagatgctggtggcggagggctgccgcgtggccagcagctacatcccggtggagaaggacctggccctgaagtggcaggccgagaacaaggcggagggcatcgacgtgttcctgaccgagggcgacgtgaccgacgcggccgactgcgagcgcatggcccaggagatcgaggacgccctgggcccgatcgacgtgctggtgaactgcgcgggcatcacccgcgacggcaccttcaagaagatggagcgcgagcagtggtacgacgtgatcgacaccaacctgaacagcgtgtacaacgtgacccgcccggtgatcaacggcatgctggagcgcaagttcggccgcgtgatcaacatctcgtcgctgaacggccgcaagggccagttcggccaggccaactacagcgcggccaaggccggcatgcacggcttcaccatggccctggcccaggaaaccgccagcaagggcatcaccgtgaacaccatctcgccgggctacatcggcaccagcatggtgatggccatcccggaggacatccgcaaccagatcatcgcgcagatcccggtgggccgcctgggccagccggacgagatcgccagcctggtggcctacctggcctcggacaagggcgccttcatcaccggcgcgaacatcgacatcaacggtggccagcacatgcactaag

SEQ ID NO: 12 - DNA, 745 bp, Artificial Sequence
  Laboratory synthesis
atgaagaagcacaccgtgctggtgaccggcggcaccggcggcatcggcaaggccatctgcatggcgctgtcggacgagggcttctcggtggtggccagctgcagcggcaactcgtgcaagaagatggacatctggcaggaagagatgaagatgcagggctacagcatcccgctggtgcgcggcgacgtggcggacttcgacagctgcaccaagatggtgcaggacgcggagcagctgatcggctcgatcgacatcctggtgaacgtggccggcatcacccgcgacggcagcttccgcaagatgagcaccacccagtggcagaacgtgatccgcaccaacctggacagcgtgtacaacgtgacccagcaggtgatcaacggcatgatcgagcgtcgcttcggccgcatcatcaacatctcgagcgtgaacggccagaagggccagttcggccagaccaactacagcgcggccaaggcgggcatgcacggcttcaccatggccctggcccaggaagtggcccacaagggcatcaccgtgaacaccgtgagcccgggctacatcgccaccgagatggtgatggcggtggacgaggacatccgcaaggagatcgtgaagcagatcccggtgggccgcttcggcgagccggaggagatcgcccgcgtggtgtcgttcctggccgacgagcagagcggcttcatcaccggcgccgacatgagcatcaacggtggcatgtacatgcactaag

SEQ ID NO: 13 - DNA, 748 bp, Artificial Sequence
  Laboratory synthesis
atggacaaggtgcaggtgtgcctggtgaccggcggcgccggcggcatcggccgcgagatctgccgtcgcatggcggccgacggctacaccgtggtggccggctgcaccagcctggacggcgccaacgccaaggccttcgcggccgagatcgagcaggaccgcctgaacatccgcctgcgcgccttcgacgtgtcggacttcgacgcgtgccagcgcaccatcatggacatcgaggagtcggtgggcagcatcgccgtgctggtgaacaacgccggcatcacccgcgacggcaccctgcgcaagatgaaccgcgcccagtgggacgaggtgctgagcgtgaacctggacagcgtgttcaacctgtcgcgcgcggtgatcaacccgatgctggagcgccagtacggccgcatcatcaacatctcgagcatcaacggccagaagggccagttcggccagtgcaactacgcggccgccaaggccgccatgtacggcttctcgaagtcgctggcccaggaaaccgccgccaagggcatcaccgtgaactgcatcagcccgggctacatcgaaaccgacatgatcctggccatcgacgaaaccatccgcgactcgatccgcaagcagatcccggtgcagcgcttcggccagccgagcgaggtggcccgcagcgtggcgttcctggccgccccggaggccggcttcatcaccggcagcaacctggcgatgaacggtggccagtacatggactaag

SEQ ID NO: 14 - DNA, 742 bp, Artificial Sequence
  Laboratory synthesis
atgaccaagcgcatcgccctggtgaccggcggcatgggcggcatcggcagcgccatctgcaaggccctggccgaggcgggccacatcgtggtgacgacctacagcaagccgggccgcgagcaggcctggcacgcggacatgaagggcctgggcttcaacgacatccactcgtaccagtgcgacgtgaccgacttcgcggcctgccaggacatcgcggcccgcatcgccaaggacatcggcccgatcagcatcctggtgaacaacgcgggcatcacccgcgacgcctcgttcaagaagcagagcaaggacgactgggacgcggtgatccgcaccaacctggactcggtgttcaacatgaccaagccggtgctggactcgatgctggaggcgggcttcggccgcatcgtgaacatctcgagcatcaacggccagaagggccagttcggccagaccaactacagcgcggccaaggccggcatgcacggcttcaccatggcgctggcccaggaagtggccaagaagggcgtgaccgtgaacaccatctcgccgggctacatcgcgaccgagatggtgatggcggtgccggaggacgtgcgcagcaagatcgtggcccagatcccggtgggccgcctgggcaagccggaggagatcgcggccctggtgggcttcctgtgcagcgagaacgcgggcttcatcaccggcagcaacatcgccatgaacggtggccagcacatgatgtaag

SEQ ID NO: 15 - DNA, 739 bp, Artificial Sequence
  Laboratory synthesis
atgaccaaccgcgtggccctggtgaccggcggcatgggcggcatcggcaacgccatctgcaaggccctgggcaaggcgggccacaccgtggtgaccacctactcgaagccgggccgcgaggacgcctgggtggccgagatgaagaccctgggcatctcggcccacgcctacccgtgcgacgtgaccgacgcggcccagtgcgcggccctggtggcgcaggtgtcgtcggagatcggcccggtggccgtgctggtgaacaacgcgggcatcacccgcgacggcaccctgcgcaagatgagcgcggaggactggtcggcggtgctggccaccaacctggacagcgtgttcttcatggcacgcccggtgatcgacggcatgctggacgcgggctggggccgcatcatcaacatctcgagcatcaacggccagaagggccagttcggccagaccaactacagcgcggccaaggccggcatgcacggcttcaccatggccctggcccaggaagtggcccgcaagggcgtgaccgtgaacaccatcagcccgggctacatcgcgaccgagatggtgatggccgtgccggaggacgtgcgcaacaagatcatcggccagatcccggtgggccgcctgggcaccccggaggagatcgccggcctggtgacctacctggccagcgacatcgccggcttcatcaccggcgccaacctgagcatcaacggtggccagcacaccatgtaag

SEQ ID NO: 16 - DNA, 739 bp, Artificial Sequence
  Laboratory synthesis
atgatcaagaccgccctgatcaccggcggcatgggcggcatcggcgagatcgtggccaagaagctgcacgacgcgggctaccgcgtgatcgtgacccactcgagccgcaacacccgcaagaagatgtggcaggcggactgcctgaaggccggctacgacttcatctgcgtggaggtggacgtggaggacatcgagtcgacccgcaagatggccaaccacatcgcggacctgggctaccacgtggacatcatcatcaacaacgccggcatcaccaaggacatcagcttcaagaagatgacctacgacgactggaacatcgtgatccgcaccaacctggactcgctgtacaacgtgaccagccagttcatcaacaagatgatcgagaagaactggggccgcgtgatcaacatctcgagcatcaacggctcgaagggccagttcggccagaccaactacgcggccagcaaggccggcgtgatcggcttcaccaagtcgctggccctggaggtggccgacaagggcatcaccgtgaactgcatctcgccgggctaccaggaaaccgccatggtgaacgcggtggacccgctgatcctgcagcagatcatcagcaccatcccgatgaagcgcctgggccagccgcgcgagatcgccgacctggtgctgtacctgtgctcggacaccagcgagttcatgaccggcgcgaacctgcacatcaacggtggccagtacatgggctaag

SEQ ID NO: 17 - DNA, 730 bp, Artificial Sequence
  Laboratory synthesis
atgagcaaggtggccctggtgaccggcggcaccggcggcatcggcagcgccgtgtgcaagcgcctggccgcggccggcttcaaggtgatcagcacctacttcgagccggaggagcaggccaaggcctgggccgagaagcaggacttcgcggtgggcctgtaccactgcaacgtgtcggactacgacagctgcgtgaagctgaagcaggccatcgaggcggacggcctgaacgtggacgtgatcgtgaacaacgccggcatcacccgcgacgcgaagttctcgaagatgacctacgacatgtggcgcgccgtgctgtcgaccaacctggacagcctgttcaacatctcgcaccagttcgtggacggcatgaccgagcgcggctggggccgcatcatcaacatctcgtcggtgaacggccagaagggccaggcgggccagaccaactactcggccgccaaggccggcgtgcacggcttcaccatggccctggcccaggaagtggtgcgcaagggcgtgaccgtgaacaccatctcgccgggctacatcggcaccgagatggtgatggccatccgcgaggacgtgcgcgagaagatcgtggcccagatcccgatgcagcgcctgggcaagccggaggagatcgccgcggtggccaacttcctggcctcggacgacgccgccttcatcaccggcgcggacttcagcgccaacggtggccagtacatgcactaag

SEQ ID NO: 18 - DNA, 775 bp, Artificial Sequence
  Laboratory synthesis
atgaccaccgacaacccgaccgcgaacaagaagatcgccctggtgaccggcgccctgggcggcatcggcaccgccatctgccacgccctgatccaggccggctaccacatcatcgccacctacacccacaaggccgacagcaccgtgaaccgcggcgaggcctggctgaaggaagagggcatgaacggctcggacttcaccttcgtggaaaccaacctgaccgaccacgaggcggccaccaaggccatcgtggacgcgatcgagaaggccggccacatcgacgtgctggtgaacaacgcgggcatcacccgcgacaccaccttcaagaagatgacctacgagcagtggtcggaggtgatcgacaccaacctgaagagcctgttcaccgtgacccagccggtgttcaacaagatgctggagcagaagtcgggccgcatcgtgagcatctcgagcatcaacggcctgaagggccagttcggccagaccaactactcggcgaccaaggccggcatcatcggcttcagcaaggccctggcccaggaaggcgccaagagcggcgtgaccgtgaacgtggtggccccgggctacaccggcaccaagatggtgatggccgtgccggagaaggtgatggagagcatcaaggcgggcatcccgatgggccgcatcgcccagccggaggagatcgcggccgccgtgatgtacctggtgtcggacggcgccgcctacatcaccggcgaaaccatcaacgtgaacggtggccagtacatgcactaag

SEQ ID NO: 19 - DNA, 742 bp, Artificial Sequence
  Laboratory synthesis
atgcagaagctggccctgatcaccggcagcaagggcggcatcggctcggccatcaccgagaagctggtgcaggacggcttccgcatcatcgcgacctacttcaccggcaactacgagtgcgccaaggagtggttcgacgagaagggcttcagcgaggaccaggtgaccctgttcgagctggacgtgaccgacgcggacagctgccgcgagcgcctgaccaagctgctggagaacgagggcaccgtggacgtgctggtgaacaacgcgggcatcacccgcgactgcaccttcaagcgcatgaccgccgagcagtggaacgacgtgatcaacaccaacctgaacagcgtgttcaacgtgacccagccgctgttcgcggccatgtgcgagaagggcggcggccgcatcatcaacatctcgagcgtgaacggcctgaagggccagttcggccagaccaactactcggccgcgaaggcgggcatgatcggcttcagcaaggccctggccttcgagggcgcccgcagcggcgtgaccgtgaacgtggtggccccgggctacaccggcaccccgatggtgcaggccatccgccaggacgtgctggacagcatcatcgaaaccgtgccgatgaagcgcctggccaccccggaggagatcgccagcgccgtggcctacctggcctcggacgccggcgcctacatcaccggcgaaaccctgagcgtgaacggcggcctgtacatgcagtaag

SEQ ID NO: 20 - DNA, 748 bp, Artificial Sequence
  Laboratory synthesis
atgacccagaagaagatcgccctggtgaccggcgcggcaggcggcatcggcaccgagatctgccgccagctggccaacaacggcttccgcgtggtggccacccaccgcccgggcaaggccgagcaggcccaggcgtggctgcaggagcagaacctggccgaccaggacatcaagctgctggccctggacgtggccgaccacgagggcgtgtcgcaggccctgggcgagctgctgaaggccgagggccgcatcgacgtgctggtgaacaacgcgggcatcacccgcgacagcgtgttcaagaagatgaccctggagcagtggcgcgacgtgatgtcgaccaacctggacagcctgttctcggtgagccagccggtgttcaacgccatgtgcgagcagggcggcggccgcatcatcaacatctcgagcgtgaacggcctgaagggccagttcggccaggtgaactactcggccgcgaaggcgggcatgatcggcttcaccaaggccctggcggccgagggcgcccgcttcggcgtgtgcgtgaacgcggtggccccgggctacaccgccaccccgatggtgaccgccatccgcgaggacgtgctggactcgatcaaggccaccatcccgctgaagcgcctggccaccaccgaggaagtggcgggcgccgtgctgtacctggcgggcgagcacggtggctacgtgaccggcgaaaccctgtcggtgaacggcggcctgtacatgcagtaag

SEQ ID NO: 21 - DNA, 748 bp, Artificial Sequence
  Laboratory synthesis
atgaccaagaaggtggccctggtgaccggcggcaccggcggcatcggcacccagatctgccgcaccctgagcaccgccggctacatcgtggtggccaactggctgaagggcatcgacgacggcccggcctgggaggcgaagcagaaggcggacggctacgacaacatcctgatcgccgagggcgacgtgagcgactacgaccaggccgtggcgatggtgaaggaagccgtggagaaggcgggcgccccgatcgacatcctggtgaacaacgccggcatcacccgcgacaagatgttccgcaagatggagaagtcgcagtgggacgcggtgatcaacagcaacctgtcgagcatcttcaacgtgaccaagcaggtgctggacggcatggtggagcgcggctggggccgcatcgtgaacatctcgtcggtgaacggccagaagggccaggcgggccaggccaactacagcgcggccaaggccggcatgcacggcttcaccatggccatcgcgcaggaagtggcctcgaagggcgtgaccgtgaacaccatcagcccgggctacatcggcaccgccatggtgatgagcatcaaggaagagatccgcaaccagatcgtggcccagatcccggtgggccgcctgggcaagccggaggagatcgcctggaccgtgcagttcctggccgacgagaagtcggcgttcatcaccggcgccaacatctcggtgaacggcggcctgcacatgggctaag

SEQ ID NO: 22 - DNA, 751 bp, Artificial Sequence
  Laboratory synthesis
atgacctcggaaaccaagcgcaccgccctggtgaccggcggcatcggcggcctgggcaccgccatcgcgcgctcgctggccgaccgcggccaccaggtgctggtggcgtactacgtgagcgacaacccgaccgagtggctggccaagcagaaggaagacggctacgacttcaaggcctacgcggtggacgtggcggacttcgagtcgtgccagcagatggtggagaagatccacgtggacggcttcaagatcgacatcctggtgaacaacgccggcatcaccaaggaccgctcgttccgcaagatgagctacgaggactgggaggcggtgctgcgcaccaacctggacagcgtgttcaacgtgaccaagcaggtgatcgacgacatgctggagtcgaagtggggccgcatcgtgaccatctcgagcgtgaacggcagcaagggccagttcggccaggccaactactcgagcgcgaagtcgggcatgtacggcttcagcaagaccctggccctggagttcgcggccaagggcatcaccgtgaacaccgtgagcccgggctacatcatgaccgagatggtggcgcagatgccgcaggagatcgtgaacgagcagatcatcccgcagatcccgatgcgtcgcctgggcaagccggaggagatcggcgagctggtggcctacatctgcagcgagtcggccggcttcatgaccggcgccaacatcgccatcaacggcggcctgcacatgtactaag

SEQ ID NO: 23 - DNA, 742 bp, Artificial Sequence
  Laboratory synthesis
atgaccgagcgcatcgccttcgtgaccggcggcatgggcggcatcggcaccgccatctgcaagcgcctggcggccaacggcaacaaggtggtggccaactgcctgccgggctacgacaagaaggacgactggctgagctcgatgcgcgcccagggctacagcgtgcacgcggccgagggcaacgtggaggagttcgactcgtgcgccgacatgttctaccgcatcggcagcatcatcggcccggtggacatcctggtgaacaacgcgggcatcacccgcgacggcgtgttcaagcgcatgtcggagagcgactggtacgacgtgatcaacaccaacctgaacagcgtgttcaacgtgacccgccaggtggtggagggcatgaccgaccgcggctggggccgcatcatcaacgtgtcgagcgtgaacgccctgaagggccagttcggccagaccaactacagcgcggccaaggccggcatgcacggcttcagcaaggccctggcccaggaagtggtgcgcaagggcgtgaccgtgaacaccatctcgccgggctacgtggccaccgagatggtgatggcgatccgcaccgaggtgcgcgaccagatcgtggccaccatcccgatgggccgcctggcccagccggacgagatcgccggcctggtggcctacctggccagcgacgacgcgggctacatcaccggcgcgaacatcagcatcaacggcggcctgcacatggcctaag

SEQ ID NO: 24 - DNA, 748 bp, Artificial Sequence
  Laboratory synthesis
atgggcagcaccagccgcatcgcggtggtgaccggcggcatgggcggcatcggcaccagcatcagccagcgcctgcacaaggaaggcttcaaggtggtggtgacctgcagcccgaactcgagccgcaagaacgactggctgccgatccagcagaaggcgggctacgacttcgagtgcgtggagatggacgtgaccgactgggagagcaccaagaacgccctgaagcaggtgcacgaggagttcggcccggtggcggtgctggtgaacaacgccggcatcacccgcgacgccagcttccgcaagctgaccccggaggactggaacgcggtgatcggcaccaacctgaccagcctgttcaacacctcgaagcaggtgctggacggcatgctggccaacggctggggccgcatcatcaacatctcgtcgatcaacggccagcgcggccagttcggccagaccaactacagcgcggccaaggccggcatccacggcttcaccatggccctggcccgcgaggtgagcggcaagggcgtgaccgtgaacaccgtgtcgccgggctacatccagaccgacatgaccgccgcgatccgccaggacatcctggacaccatgatcgcggccaccccggtgggccgcctgggccgtccggaggagatcgccagcatcgtggcctggctggccagcgaggagtcggcctacagcaccggcgccgacttctcgatcaacggtggcatgaacatgcagtaag

SEQ ID NO: 25 - DNA, 748 bp, Artificial Sequence
  Laboratory synthesis
atgaccgacagcgcccgcatcgccctggtgaccggcggcatgggcggcatcggcaccgccatctcgcagcgcctgcaccgcgagggcttcaccgtggtggtgggctgcagcccggccagcagccgcaagaacgactggatcagccgccagcaggaagccggctaccacttccactgcgtggactgcgacatcaccgactgggagagcacccgccagggcttcgagctggtgcgcgagtcggtgggcccgatcgacgtgctggtgaacaacgcgggcatcacccgcgacgccaccttccgcaagctgaccccggagaactggcgcgccgtgatcgaaaccaacctgaacggcctgttcaacaccaccaagcaggtgatcgacagcatgctggcccgcaactggggccgcatcatcaacatctcgtcgatcaacggccagcgcggccagttcggccagaccaactactcggcggccaaggcgggcatccacggcttcaccatggccctggcccgcgaggtgtcgggcaagggcgtgaccgtgaacaccgtgagcccgggctacatccagaccgacatgaccgcggccatccgcccggacatcctggagggcatgatcgcgggcatcccggtgggccgcctgggccagccggaggagatcgccagcatcgtggcctggctggccagcaccgagtcggcctacgccaccggcgccgacttctcggtgaacggtggcatgaacatgcagtaag

SEQ ID NO: 26 - DNA, 748 bp, Artificial Sequence
  Laboratory synthesis
atgaacaccgagaaccagcacatcgccctggtgaccggcgccaccggcggcctgggcacccacatctgcaagcgcctgtcggaggacggctacatcgtgtgcgccaactaccgcagcgaggagaaggcgcaggagtggaagaagaagatggaggccgagggctaccagttctacctgtacaaggcggacgtgtgcgactacgacgccgtggagcagatgatcaaggcgatcgagcaggaccacggcgtggtggacatcctggtgaacaacgccggcatcaccaaggacggcatcttcaagaagatgtcgaaggagaactggcaggacgtgatcgcgaccaacctgaccagcgtgttcaactgctgccgccacgtgatcaaccagatgatcgaccagaattacggccgcatcgtgaacatctcgtcggtgaacggccagcgcgcccagttcggccaggtgaactacgcggccgccaaggccggcatgcacggcatcaccaagaccctggcgatcgaggtggccaacaagggcatcaccgtgaacaccatctcgccgggctacgtggcgaccgacatggtgatggccgtgccggaggaagtgcgcaacaagatcatcgcgggcatcccggtgggccgcctgggcggcaccggcgagatcgcccacctggtgagcttcctggccgcccgcgacaccgccttcatcaccggcgcgaactacgccatcaacggtggccagcacgtgtactaag

SEQ ID NO: 27 - DNA, 745 bp, Artificial Sequence
  Laboratory synthesis
atgaccaagcgcatcgcggtggtgaccggcggcatgggcggcctgggcgaggcggtgtcgatccgcctgaacgacgcgggccaccgcgtggtggtgacctacagcccgagcaacaccggcgccgaccgctggctgaccgagatgcacgccaccggccgcgagttccacgcctacccggtggacgtggcggaccacgacagctgccagcagtgcatcgagaagatcgcccgcgacgtgggcccggtggacatcctggtgaacaacgcgggcatcacccgcgacatgaccctgcgcaagctggacaaggtgaactgggacgcggtgatccgcaccaacctggactcggtgttcaacatgaccaagccggtgtgcgagagcatggtggagcgcggctggggccgcatcgtgaacatctcgtcggtgaacggcagcaagggctcggtgggccagaccaactacgcggccgccaaggcgggcatgcacggcttcaccaagagcctggccctggagatcgcccgcaagggcgtgaccgtgaacaccgtgagcccgggctacctggcgaccaagatggtgaccgccatcccgcaggacatcctggactcgaagatcctgccgcagatcccggccggccgcctgggcaagccggaggaagtggccgccctggtggcctacctgtgcagcgaggaagccggcttcgtgaccggcagcaacatcgccatcaacggtggccagcacatgcactaag

SEQ ID NO: 28 - DNA, 742 bp, Artificial Sequence
  Laboratory synthesis
atgctgcgcgtggccctggtgaccggcggcatgggcggcctgggcgaggcgatctgcatcaagctggccgcgctgggctacaaggtggtgaccacctactcgccgagcaacaccaaggcccacgagtggctgcgcaccatgaacgacatgggctacggcttcaaggcctacccgtgcgacgtgggcgacttcgactcgtgcaaggcgtgcgtggagcaggtgagcaaggacgtgggcgcggtggaggtgctggtgaacaacgcgggcatcacccgcgacatgaccttcaagaagatgaccaaggccgactgggacgcggtgatccacaccaacctggactcgtgcttcaacatgaccaagcaggtgatggacggcatgatggagcgcggctggggccgcgtgatcaacatctcgtcggtgaacggccagaagggcgccttcggccagaccaactacagcgcggccaaggccggcatgcacggcttcaccaaggccctggccctggaggtggccaagaagggcgtgaccgtgaacaccatcagcccgggctacatcggcaccaagatggtgatggcgatcccgcaggaagtgctggagtcgaagatcctgccgcagatcccgcagtcgcgcctgggcaagccggaggaagtggcgggcctggtggcctacctgagctcggaggaagccgccttcgtgaccggcgccaacatcagcatcaacggtggccagcacatgtactaag

SEQ ID NO: 29 - protein, 593 aa, Artificial Sequence
  Laboratory synthesis
MSQPSYGPLFEALAHYNDKLLAMAKAQTERTAQALLQTNLDDLGQVLEQGSQQPWQLIQAQMNWWQDQLKLMQHTLLKSAGQPSEPVITPERSDRRFKAEAWSEQPIYDYLKQSYLLTARHLLASVDALEGVPQKSRERLRFFTRQYVSAMAPSNFLATNPELLKLTLESGGQNLVRGLALLAEDLERSADQLNIRLTDESAFELGRDLALTPGRVVQRTELYELIQYSPTTETVGKTPVLIVPPFINKYYIMDMRPQNSLVAWLVAQGQTVFMISWRNPGVAQAQIDLDDYVVDGVIAALDGVEAATGEREVHGIGYCIGGTALSLAMGWLAARRQKQRVRTATLFTTLLDFSQPGELGIFIHEPIIAALEAQNEAKGIMDGRQLAVSFSLLRENSLYWNYYIDSYLKGQSPVAFDLLHWNSDSTNVAGKTHNSLLRRLYLENQLVKGELKIRNTRIDLGKVKTPVLLVSAVDDHIALWQGTWQGMKLFGGEQRFLLAESGHIAGIINPPAANKYGFWHNGAEAESPESWLAGATHQGGSWWPEMMGFIQNRDEGSEPVPARVPEEGLAPAPGHYVKVRLNPVFACPTEEDA

SEQ ID NO: 30 - DNA, 146 bp, Artificial Sequence
  Laboratory synthesis
atgcctccacaccgctcgtcacatcctgttgcgttcactggaatcccacgatagagtttgacctgcgagcaagctgtcaccggatgtgctttccggtctgatgagtccgtgaggacgaaacagcctctacaaataattttgtttaa

SEQ ID NO: 31 - protein, 246 aa, Artificial Sequence
  Laboratory synthesis
MTQRIAYVTGGMGGIGTAICQRLAKDGFRVVAGCGPNSPRREKWLEQQKALGFDFIASEGNVADWDSTKTAFDKVKSEVGEVDVLINNAGITRDVVFRKMTRADWDAVIDTNLTSLFNVTKQVIDGMADRGWGRIVNISSVNGQKGQFGQTNYSTAKAGLHGFTMALAQEVATKGVTVNTVSPGYIATDMVKAIRQDVLDKIVATIPVKRLGLPEEIASICAWLSSEESGFSTGADFSLNGGLHMG

SEQ ID NO: 32 - DNA, 20 bp, Artificial Sequence
  Laboratory synthesis
gcagacttggccgggtacca

SEQ ID NO: 33 - DNA, 19 bp, Artificial Sequence
  Laboratory synthesis
caccgctcgtcacatcctg

SEQ ID NO: 34 - DNA, 40 bp, Artificial Sequence
  Laboratory synthesis
tggtacccggccaagtctgcgggcgtgcccatgatgtaga

SEQ ID NO: 35 - DNA, 42 bp, Artificial Sequence
  Laboratory synthesis
tgagacccaaggtctccatgatttgattgtctctctgccgtc

SEQ ID NO: 36 - DNA, 38 bp, Artificial Sequence
  Laboratory synthesis
ggagaccttgggtctcagtgacgcttgcatgagtgccg

SEQ ID NO: 37 - DNA, 39 bp, Artificial Sequence
  Laboratory synthesis
caggatgtgacgagcggtgcatggtgtcgaccagcttgg

SEQ ID NO: 38 - DNA, 11 bp, Artificial Sequence
  Laboratory synthesis
gtgaagagacc

SEQ ID NO: 39 - DNA, 21 bp, Artificial Sequence
  Laboratory synthesis
tggtctggctggcggactgag

SEQ ID NO: 40 - DNA, 21 bp, Artificial Sequence
  Laboratory synthesis
ggcgaactcatcctgcgcctc

SEQ ID NO: 41 - DNA, 24 bp, Artificial Sequence
  Laboratory synthesis
catgatttgattgtctctctgccg

SEQ ID NO: 42 - DNA, 20 bp, Artificial Sequence
  Laboratory synthesis
gtgacgcttgcatgagtgcc

SEQ ID NO: 43 - DNA, 39 bp, Artificial Sequence
  Laboratory synthesis
agagagacaatcaaatcatgactcagcgcattgcgtatg

SEQ ID NO: 44 - DNA, 40 bp, Artificial Sequence
  Laboratory synthesis
ggcactcatgcaagcgtcactcagcccatatgcaggccgc

SEQ ID NO: 45 - DNA, 39 bp, Artificial Sequence
  Laboratory synthesis
tggtacccggccaagtctgtgtggaactacgtggtcgac

SEQ ID NO: 46 - DNA, 42 bp, Artificial Sequence
  Laboratory synthesis
tgagacccaaggtctccattcatgccttggctttgacgtatc

SEQ ID NO: 47 - DNA, 40 bp, Artificial Sequence
  Laboratory synthesis
gctgggccgccgaagtgagcttcgacggcgtcttcgttcc

SEQ ID NO: 48 - DNA, 38 bp, Artificial Sequence
  Laboratory synthesis
cgagcggtgtggaggcatctattcagtcagggatgcct

SEQ ID NO: 49 - DNA, 43 bp, Artificial Sequence
  Laboratory synthesis
ctacaaataattttgtttaactgactgaataggaagagcaagc

SEQ ID NO: 50 - DNA, 41 bp, Artificial Sequence
  Laboratory synthesis
ccctgatttccataaggcgccgcacgccgcgcggtgacgac

SEQ ID NO: 51 - DNA, 18 bp, Artificial Sequence
  Laboratory synthesis
ttcgtggtctcggccgat

SEQ ID NO: 52 - DNA, 19 bp, Artificial Sequence
  Laboratory synthesis
caaagtcactgggttcccg